European Patent Specification EP 4 347 887 B1, published December 24, 2025. Title: Biomarker. Applicant: Panagiotis Ntostis. The sequence listing filed with the application follows.

SEQUENCE LISTING (56 sequences)

SEQ ID NO: 1 - DNA, 20 bp, Artificial Sequence
  ACTB Primer (Forward)
aagccaccccacttctctct

SEQ ID NO: 2 - DNA, 20 bp, Artificial Sequence
  ACTB Primer (Reverse)
ctatcacctcccctgtgtgg

SEQ ID NO: 3 - DNA, 20 bp, Artificial Sequence
  BAK1 Primer (Forward)
ttcaccaagattgccaccag

SEQ ID NO: 4 - DNA, 20 bp, Artificial Sequence
  BAK1 Primer (Reverse)
atgctggtagacgtgtaggg

SEQ ID NO: 5 - DNA, 20 bp, Artificial Sequence
  BRAP Primer (Forward)
tgactgaactccccaagtgc

SEQ ID NO: 6 - DNA, 20 bp, Artificial Sequence
  BRAP Primer (Reverse)
ggcaaacaggacacgtggta

SEQ ID NO: 7 - DNA, 20 bp, Artificial Sequence
  CCPG1 Primer (Forward)
ccccgagtgctataccgaac

SEQ ID NO: 8 - DNA, 25 bp, Artificial Sequence
  CCPG1 Primer (Reverse)
cagacatctttcaggtcatatggat

SEQ ID NO: 9 - DNA, 23 bp, Artificial Sequence
  DAB2 Primer (Forward)
ctagctattgcaaatgagggaag

SEQ ID NO: 10 - DNA, 26 bp, Artificial Sequence
  DAB2 Primer (Reverse)
ggtaatactacttgaacccaggagca

SEQ ID NO: 11 - DNA, 22 bp, Artificial Sequence
  DBI Primer (Forward)
gctgcgaagtgtagacccttgt

SEQ ID NO: 12 - DNA, 21 bp, Artificial Sequence
  DBI Primer (Reverse)
atggcttggtcttaaggtgcc

SEQ ID NO: 13 - DNA, 20 bp, Artificial Sequence
  FABP3 Primer (Forward)
cgcctgctctcttgtagctt

SEQ ID NO: 14 - DNA, 22 bp, Artificial Sequence
  FABP3 Primer (Reverse)
atatgagcgagtgacttcatgt

SEQ ID NO: 15 - DNA, 23 bp, Artificial Sequence
  GAPDH Primer (Forward)
ttgtcaagctcatttcctggtat

SEQ ID NO: 16 - DNA, 23 bp, Artificial Sequence
  GAPDH Primer (Reverse)
tctctcttcctcttgtgctcttg

SEQ ID NO: 17 - DNA, 20 bp, Artificial Sequence
  H3F3B Primer (Forward)
tgctggtttttcgctcgtcg

SEQ ID NO: 18 - DNA, 22 bp, Artificial Sequence
  H3F3B Primer (Reverse)
gccattttctttcacccaacgc

SEQ ID NO: 19 - DNA, 20 bp, Artificial Sequence
  HNRNPC Primer (Forward)
gccagcaacgttaccaacaa

SEQ ID NO: 20 - DNA, 20 bp, Artificial Sequence
  HNRNPC Primer (Reverse)
tgaacagagcagcccacaat

SEQ ID NO: 21 - DNA, 22 bp, Artificial Sequence
  IFITM3 Primer (Forward)
ctgggcttcatagcattcgcct

SEQ ID NO: 22 - DNA, 22 bp, Artificial Sequence
  IFITM3 Primer (Reverse)
agatgttcaggcacttggcggt

SEQ ID NO: 23 - DNA, 21 bp, Artificial Sequence
  ZFAND5 Primer (Forward)
gtccatcagtttctcagccca

SEQ ID NO: 24 - DNA, 21 bp, Artificial Sequence
  ZFAND5 Primer (Reverse)
ggcagtcaaaccctgtaagac

SEQ ID NO: 25 - DNA, 21 bp, Artificial Sequence
  ACAT2 Primer (Forward)
gcggaccatcataggttcctt

SEQ ID NO: 26 - DNA, 20 bp, Artificial Sequence
  ACAT2 Primer (Reverse)
tgctgccaagacatgtccaa

SEQ ID NO: 27 - DNA, 21 bp, Artificial Sequence
  FABP5 Primer (Forward)
catgaaggagctaggagtggg

SEQ ID NO: 28 - DNA, 22 bp, Artificial Sequence
  FABP5 Primer (Reverse)
cccagggtacaagaaaactgtg

SEQ ID NO: 29 - DNA, 20 bp, Artificial Sequence
  HINT1 Primer (Forward)
ttgaggatgaccggtgcctt

SEQ ID NO: 30 - DNA, 21 bp, Artificial Sequence
  HINT1 Primer (Reverse)
agcagcacatttcttgccaac

SEQ ID NO: 31 - DNA, 20 bp, Artificial Sequence
  HSP90AA1 Primer (Forward)
cgtttctgagaagcagggca

SEQ ID NO: 32 - DNA, 20 bp, Artificial Sequence
  HSP90AA1 Primer (Reverse)
gggaatgcagagacgtggaa

SEQ ID NO: 33 - DNA, 20 bp, Artificial Sequence
  IFITM3 Primer (Forward)
cgcctactccgtgaagtcta

SEQ ID NO: 34 - DNA, 21 bp, Artificial Sequence
  IFITM3 Primer (Reverse)
ccataggcctggaagatcagc

SEQ ID NO: 35 - DNA, 18 bp, Artificial Sequence
  LRP2 Primer (Forward)
cgtcgcggagatggatcg

SEQ ID NO: 36 - DNA, 20 bp, Artificial Sequence
  LRP2 Primer (Reverse)
cgcactgtcacattcttggc

SEQ ID NO: 37 - DNA, 20 bp, Artificial Sequence
  PEBP1 Primer (Forward)
caccagcatttcgtgggatg

SEQ ID NO: 38 - DNA, 23 bp, Artificial Sequence
  PEBP1 Primer (Reverse)
caggaaatgatgccattctctgt

SEQ ID NO: 39 - DNA, 20 bp, Artificial Sequence
  PRDX5 Primer (Forward)
ggatgttccaaggttcggct

SEQ ID NO: 40 - DNA, 20 bp, Artificial Sequence
  PRDX5 Primer (Reverse)
agggccttcactatgccatc

SEQ ID NO: 41 - DNA, 19 bp, Artificial Sequence
  PSMA5 Primer (Forward)
ttagtactgcggccgtgtg

SEQ ID NO: 42 - DNA, 21 bp, Artificial Sequence
  PSMA5 Primer (Reverse)
agtattcacgcccctgtcgta

SEQ ID NO: 43 - DNA, 16 bp, Artificial Sequence
  TAGLN2 Primer (Forward)
gcttgaacgctccccg

SEQ ID NO: 44 - DNA, 20 bp, Artificial Sequence
  TAGLN2 Primer (Reverse)
tccactggatcaggatctgc

SEQ ID NO: 45 - DNA, 20 bp, Artificial Sequence
  PRDX2 Primer (Forward)
cgagcatggggaagtttgtc

SEQ ID NO: 46 - DNA, 20 bp, Artificial Sequence
  PRDX2 Primer (Reverse)
ggcacaagctcactatccgt

SEQ ID NO: 47 - DNA, 20 bp, Artificial Sequence
  ATG3 Primer (Forward)
ccccaggatgcagaatgtga

SEQ ID NO: 48 - DNA, 20 bp, Artificial Sequence
  ATG3 Primer (Reverse)
tccagctgccacaaactctt

SEQ ID NO: 49 - DNA, 20 bp, Artificial Sequence
  MCL1 Primer (Forward)
aacaaagaggctgggatggg

SEQ ID NO: 50 - DNA, 20 bp, Artificial Sequence
  MCL1 Primer (Reverse)
tgccaaaccagctcctactc

SEQ ID NO: 51 - DNA, 18 bp, Artificial Sequence
  MTMR14 Primer (Forward)
cggcggctctaaggttga

SEQ ID NO: 52 - DNA, 19 bp, Artificial Sequence
  MTMR14 Primer (Reverse)
gatgtgccggggatagtgg

SEQ ID NO: 53 - DNA, 19 bp, Artificial Sequence
  PI4KB Primer (Forward)
gggtcccccagaggatcaa

SEQ ID NO: 54 - DNA, 20 bp, Artificial Sequence
  PI4KB Primer (Reverse)
caaaacttgctccggccttc

SEQ ID NO: 55 - DNA, 17 bp, Artificial Sequence
  PPP1R15A Primer (Forward)
gcttgaacgctccccgc

SEQ ID NO: 56 - DNA, 19 bp, Artificial Sequence
  PPP1R15A Primer (Reverse)
atcctttcggcactgggtg